European Patent Application EP 4 663 750 A1, published December 17, 2025. Title: Cell that can differentiate into M2 macrophage in tumor tissue and then expresses inflammatory cytokine after differentiation into M2 macrophage, and composition comprising the same. Applicant: Kyushu University. The sequence listing filed with the application follows.

SEQUENCE LISTING (32 sequences)

SEQ ID NO: 1 - DNA, 22 bp, synthetic construct
  source 1..22: mol_type = other DNA
cccagcaaggacactgagcaag

SEQ ID NO: 2 - DNA, 24 bp, synthetic construct
  source 1..24: mol_type = other DNA
ggtctgggatggaaattgtgaggg

SEQ ID NO: 3 - DNA, 20 bp, synthetic construct
  source 1..20: mol_type = other DNA
cagaagaatggaagagtcag

SEQ ID NO: 4 - DNA, 20 bp, synthetic construct
  source 1..20: mol_type = other DNA
cagatatgcagggagtcacc

SEQ ID NO: 5 - DNA, 22 bp, synthetic construct
  source 1..22: mol_type = other DNA
gtctcctctgacttcaacagcg

SEQ ID NO: 6 - DNA, 22 bp, synthetic construct
  source 1..22: mol_type = other DNA
accaccctgttgctgtagccaa

SEQ ID NO: 7 - DNA, 19 bp, synthetic construct
  source 1..19: mol_type = other DNA
gagcatggatcgcctacag

SEQ ID NO: 8 - DNA, 21 bp, synthetic construct
  source 1..21: mol_type = other DNA
cagacggtaacggacgtaatc

SEQ ID NO: 9 - DNA, 23 bp, synthetic construct
  source 1..23: mol_type = other DNA
gcatagccaagaccttctcctac

SEQ ID NO: 10 - DNA, 22 bp, synthetic construct
  source 1..22: mol_type = other DNA
acgtgccttctggcatcttctg

SEQ ID NO: 11 - DNA, 22 bp, synthetic construct
  source 1..22: mol_type = other DNA
accttcctgctcgcctagtgtt

SEQ ID NO: 12 - DNA, 22 bp, synthetic construct
  source 1..22: mol_type = other DNA
ggctacagagaatgacgttggc

SEQ ID NO: 13 - DNA, 22 bp, synthetic construct
  source 1..22: mol_type = other DNA
tgtggcaccaagtacctgctca

SEQ ID NO: 14 - DNA, 22 bp, synthetic construct
  source 1..22: mol_type = other DNA
gcaccttgatgaggttggactc

SEQ ID NO: 15 - DNA, 22 bp, synthetic construct
  source 1..22: mol_type = other DNA
gatacggcactggctacttcca

SEQ ID NO: 16 - DNA, 21 bp, synthetic construct
  source 1..21: mol_type = other DNA
gccagacagttttcctccgcc

SEQ ID NO: 17 - DNA, 24 bp, synthetic construct
  source 1..24: mol_type = other DNA
gtggagaatacaaatgtcagcacc

SEQ ID NO: 18 - DNA, 22 bp, synthetic construct
  source 1..22: mol_type = other DNA
ctccatcaccacctcagcagag

SEQ ID NO: 19 - DNA, 22 bp, synthetic construct
  source 1..22: mol_type = other DNA
caacagccacaaccgttacacc

SEQ ID NO: 20 - DNA, 22 bp, synthetic construct
  source 1..22: mol_type = other DNA
cttggatcagcaccgcctcttt

SEQ ID NO: 21 - DNA, 23 bp, synthetic construct
  source 1..23: mol_type = other DNA
gagtaactctggaacttggaggc

SEQ ID NO: 22 - DNA, 22 bp, synthetic construct
  source 1..22: mol_type = other DNA
atggactcctccacgaagatgc

SEQ ID NO: 23 - DNA, 22 bp, synthetic construct
  source 1..22: mol_type = other DNA
gcagtcttccagaagtaaccgc

SEQ ID NO: 24 - DNA, 23 bp, synthetic construct
  source 1..23: mol_type = other DNA
gctctcctctgttccaatactgc

SEQ ID NO: 25 - DNA, 22 bp, synthetic construct
  source 1..22: mol_type = other DNA
gattctgtgcccacagtaaggc

SEQ ID NO: 26 - DNA, 22 bp, synthetic construct
  source 1..22: mol_type = other DNA
tggtcacagagccaccttcttg

SEQ ID NO: 27 - DNA, 22 bp, synthetic construct
  source 1..22: mol_type = other DNA
gatgctgtcactaccgtgggaa

SEQ ID NO: 28 - DNA, 22 bp, synthetic construct
  source 1..22: mol_type = other DNA
caatgccagatggcaaggttgg

SEQ ID NO: 29 - DNA, 23 bp, synthetic construct
  source 1..23: mol_type = other DNA
gtgcctcaagaaatgtgccactg

SEQ ID NO: 30 - DNA, 22 bp, synthetic construct
  source 1..22: mol_type = other DNA
ggagtggtcttcagaatcctgc

SEQ ID NO: 31 - DNA, 1446 bp, Homo sapiens
  source 1..1446: mol_type = genomic DNA
ggcgcatgccatcacacccggccaatttttgtatttttggtagagatggggtttctccatgttggccaggctggtcttgaactcctgacctcaggtgatccacctgcctgggccttccaaagtgctgggattacagtcatgaatcactgcacccagcccatgtgttctgagcacccaacatgtgcctgatcctcagagggccctgggaatgccaagaaaaatgaagggagaccccagcctcctagagcttggagtctgacttctagggaggggcttgagaaagagaaaacctgacccagtctgctcagggccacattccaggtcccctagaaggctttgaagtcctgagagggtgtgcttaccaaggacatgacatttcaaacagctttgacgcataagtaggagtttatgtggtagagatgtggaaagtgacattaaaggccagggacaggccgcagtcccttttgaggaagtgtgaggagtgtggtgtgatccctcaggggaaggagaccagtggggaaaggcctgtccggaaacggggccttgaaggccacagacaggagcccgggacctgcctttaggtgaatggggagccacggcagggttctgaagcaggagagagagtgtgtagctctggaccactcacgctggctgctgcagggtggggatggcattgaggaggccagcatcccagcctgaggtggaggtggcctggactgggcaggaacagtggggttggagagaaggagcagatctgagagagatttaggaagcagaatcaacgggacatggacatggtgagggactgagacaggagtgggggagggagagcccggcagccactgggaaggaagatcaggcaggacagaagtgtgggtagatgctttccataaaccgttgagaaatccacgacctggcccaaatgtggacttcacgagaagccccagatgggtcaatgggtccataggcctctcccattgaagagagaccagtaatgccgtcattaagggtacaagacaggcctcaattctaggtgagggttggtccacgttctcacttgatttacaaccagtgaagtcaacagagctgtgaaaccatctcccccatttccagatggggaaaccaagtcccagagacacccagacatggccaaggccacacagtgcagagaccctggggagcacaagcctctaagagggggattttacaagtctgtctgaaaccagaggcgaggacagagttgagggggggtcccctctgagtggttccccgccaaagagaatttctccactttggaggaagtgggaggtagttcttcttttgagatgtgaatgtcaagtgactctgggcaccccggtgactaagaggtaagtaagtgaggcttgtgggtggagccagcaccttaaatagcaggtcttcctatgtccctttgcagacacctgggct

SEQ ID NO: 32 - DNA, 759 bp, Homo sapiens
  source 1..759: mol_type = other DNA
atgtacaggatgcaactcctgtcttgcattgcactaagtcttgcacttgtcacaaacagttcaactgaatccatgataagagacgtagaacttgccgaagaagccctccccaaaaagacaggtggcccccaaggaagtcggaggtgcctgttcctgtcacttttttcatttcttatagtggccggtgctacaaccttgttctgtctcctgcactttggtgtgatcggtccccaacgagaagagtttcctcgagacctttccctgataagccccttggcccaggccgtgaggtcatctagtaggacaccaagcgataagcctgtagcacatgtcgttgccaacccccaagcagaaggacagctccagtggctgaaccggcgagctaatgcattgttggctaacggagtagaacttcgagataaccaactcgtagttccatccgaaggtttgtacttgatttattcccaagttctttttaaggggcaaggttgtccctcaacccacgtattgttgactcatacaatatcacgaatagctgttagctatcaaacaaaagtaaatttgctttccgctatcaagtctccttgtcaacgggaaactccagagggcgccgaagctaaaccttggtacgagcccatttacctcgggggcgtcttccaactggaaaagggggaccgcttgtctgccgagatcaaccggcccgattatttggattttgccgagagtgggcaggtgtattttggcatcattgctctctaa